European Patent Specification EP 3 669 944 B1, published December 20, 2023. Title: USE OF AKKERMANSIA IN THE TREATMENT OF ORAL DISEASES. Applicant: A-MANSIA BIOTECH CANI, Patrice DE VOS, Willem AMAR, Salomon. The sequence listing filed with the application follows.

SEQUENCE LISTING (2 sequences)

SEQ ID NO: 1 - protein, 286 aa, Akkermansia muciniphila
  AMUC_1100
IVNSKRSELDKKISIAAKEIKSANAAEITPSRSSNEELEKELNRYAKAVGSLETAYKPFLASSALVPTTPTAFQNELKTFRDSLISSCKKKNILITDTSSWLGFQVYSTQAPSVQAASTLGFELKAINSLVNKLAECGLSKFIKVYRPQLPIETPANNPEESDEADQAPWTPMPLEIAFQGDRESVLKAMNAITGMQDYLFTVNSIRIRNERMMPPPIANPAAAKPAAAQPATGAASLTPADEAAAPAAPAIQQVIKPYMGKEQVFVQVSLNLVHFNQPKAQEPSE

SEQ ID NO: 2 - protein, 316 aa, Akkermansia muciniphila
  AMUC_1100 with signal peptide
MSNWITDNKPAAMVAGVGLLLFLGLSATGYIVNSKRSELDKKISIAAKEIKSANAAEITPSRSSNEELEKELNRYAKAVGSLETAYKPFLASSALVPTTPTAFQNELKTFRDSLISSCKKKNILITDTSSWLGFQVYSTQAPSVQAASTLGFELKAINSLVNKLAECGLSKFIKVYRPQLPIETPANNPEESDEADQAPWTPMPLEIAFQGDRESVLKAMNAITGMQDYLFTVNSIRIRNERMMPPPIANPAAAKPAAAQPATGAASLTPADEAAAPAAPAIQQVIKPYMGKEQVFVQVSLNLVHFNQPKAQEPSE